European Patent Specification EP 3 723 782 B1, published December 3, 2025. Title: PEPTIDES FOR TREATMENT AND PREVENTION OF NONALCOHOLIC FATTY LIVER DISEASE AND FIBROSIS. Applicant: Université de Strasbourg et al. The sequence listing filed with the application follows.

SEQUENCE LISTING (52 sequences)

SEQ ID NO: 1 - protein, 672 aa, Homo sapiens
MADVFPGNDSTASQDVANRFARKGALRQKNVHEVKDHKFIARFFKQPTFCSHCTDFIWGFGKQGFQCQVCCFVVHKRCHEFVTFSCPGADKGPDTDDPRSKHKFKIHTYGSPTFCDHCGSLLYGLIHQGMKCDTCDMNVHKQCVINVPSLCGMDHTEKRGRIYLKAEVADEKLHVTVRDAKNLIPMDPNGLSDPYVKLKLIPDPKNESKQKTKTIRSTLNPQWNESFTFKLKPSDKDRRLSVEIWDWDRTTRNDFMGSLSFGVSELMKMPASGWYKLLNQEEGEYYNVPIPEGDEEGNMELRQKFEKAKLGPAGNKVISPSEDRKQPSNNLDRVKLTDFNFLMVLGKGSFGKVMLADRKGTEELYAIKILKKDVVIQDDDVECTMVEKRVLALLDKPPFLTQLHSCFQTVDRLYFVMEYVNGGDLMYHIQQVGKFKEPQAVFYAAEISIGLFFLHKRGIIYRDLKLDNVMLDSEGHIKIADFGMCKEHMMDGVTTRTFCGTPDYIAPEIIAYQPYGKSVDWWAYGVLLYEMLAGQPPFDGEDEDELFQSIMEHNVSYPKSLSKEAVSVCKGLMTKHPAKRLGCGPEGERDVREHAFFRRIDWEKLENREIQPPFKPKVCGKGAENFDKFFTRGQPVLTPPDQLVIANIDQSDFEGFSYVNPQFVHPILQSAV

SEQ ID NO: 2 - protein, 257 aa, Homo sapiens
FNFLMVLGKGSFGKVMLADRKGTEELYAIKILKKDVVIQDDDVECTMVEKRVLALLDKPPFLTQLHSCFQTVDRLYFVMEYVNGGDLMYHIQQVGKFKEPQAVFYAAEISIGLFFLHKRGIIYRDLKLDNVMLDSEGHIKIADFGMCKEHMMDGVTTRTFCGTPDYIAPEIIAYQPYGKSVDWWAYGVLLYEMLAGQPPFDGEDEDELFQSIMEHNVSYPKSLSKEAVSVCKGLMTKHPAKRLGCGPEGERDVREHA

SEQ ID NO: 3 - protein, 12 aa, artificial sequence
  segment of kinase domain of alphaPKC
VECTMVEKRVLA

SEQ ID NO: 4 - protein, 8 aa, artificial sequence
  segment of kinase domain of alphaPKC
LMYHIQQV

SEQ ID NO: 5 - protein, 4 aa, artificial sequence
  segment of kinase domain of alphaPKC
PEII

SEQ ID NO: 6 - protein, 16 aa, artificial sequence
  segment of kinase domain of alphaPKC
SVDWWAYGVLLYEMLA

SEQ ID NO: 7 - protein, 12 aa, artificial sequence
  segment of kinase domain of alphaPKC
EDEDELFQSIME

SEQ ID NO: 8 - protein, 7 aa, artificial sequence
  segment of kinase domain of alphaPKC
GERDVRE

SEQ ID NO: 9 - protein, 12 aa, artificial sequence
  mutated segment of kinase domain of alphaPKC
  MISC_FEATURE (5)..(5): Xaa is any amino acid except R, M and P
VECTXVEKRVLA

SEQ ID NO: 10 - protein, 12 aa, artificial sequence
  mutated segment of kinase domain of alphaPKC
  MISC_FEATURE (9)..(9): Xaa is any amino acid except M, P and R
VECTMVEKXVLA

SEQ ID NO: 11 - protein, 12 aa, artificial sequence
  mutated segment of kinase domain of alphaPKC
  MISC_FEATURE (5)..(5): Xaa is any amino acid except M, P and R
  MISC_FEATURE (9)..(9): Xaa is any amino acid except M, P and R
VECTXVEKXVLA

SEQ ID NO: 12 - protein, 8 aa, artificial sequence
  mutated segment of kinase domain of alphaPKC
  MISC_FEATURE (2)..(2): Xaa is any amino acid except M, P and R
LXYHIQQV

SEQ ID NO: 13 - protein, 16 aa, artificial sequence
  mutated segment of kinase domain of alphaPKC
  MISC_FEATURE (14)..(14): Xaa is any amino acid except M, P and R
SVDWWAYGVLLYEXLA

SEQ ID NO: 14 - protein, 12 aa, artificial sequence
  mutated segment of kinase domain of alphaPKC
  MISC_FEATURE (11)..(11): Xaa is any amino acid except M, P and R
EDEDELFQSIXE

SEQ ID NO: 15 - protein, 7 aa, artificial sequence
  mutated segment of kinase domain of alphaPKC
  MISC_FEATURE (3)..(3): Xaa is any amino acid except M, P and R
GEXDVRE

SEQ ID NO: 16 - protein, 7 aa, artificial sequence
  mutated segment of kinase domain of alphaPKC
  MISC_FEATURE (6)..(6): Xaa is any amino acid except M, P and R
GERDVXE

SEQ ID NO: 17 - protein, 7 aa, artificial sequence
  mutated segment of kinase domain of alphaPKC
  MISC_FEATURE (3)..(3): Xaa is any amino acid except M, P and R
  MISC_FEATURE (6)..(6): Xaa is any amino acid except M, P and R
GEXDVXE

SEQ ID NO: 18 - protein, 4 aa, artificial sequence
  mutated segment of kinase domain of alphaPKC
  MISC_FEATURE (1)..(1): Xaa is any amino acid except M, P and R
XEII

SEQ ID NO: 19 - protein, 12 aa, artificial sequence
  mutated segment of kinase domain of alphaPKC
VECTTVEKEVLA

SEQ ID NO: 20 - protein, 25 aa, artificial sequence
  mutated segment of kinase domain of alphaPKC
  MISC_FEATURE (5)..(5): Xaa is any amino acid except M, P and R
  MISC_FEATURE (9)..(9): Xaa is any amino acid except M, P and R
  MISC_FEATURE (17)..(18): Xaa is any amino acid except M, P and R
VECTXVEKXVLALLDKXXFLTQLHS

SEQ ID NO: 21 - protein, 25 aa, artificial sequence
  mutated segment of kinase domain of alphaPKC
  MISC_FEATURE (17)..(18): Xaa is any amino acid except M, P and R
VECTMVEKRVLALLDKXXFLTQLHS

SEQ ID NO: 22 - protein, 25 aa, artificial sequence
  mutated segment of kinase domain of alphaPKC
  MISC_FEATURE (5)..(5): Xaa is any amino acid except M, P and R
VECTXVEKRVLALLDKPPFLTQLHS

SEQ ID NO: 23 - protein, 25 aa, artificial sequence
  mutated segment of kinase domain of alphaPKC
  MISC_FEATURE (9)..(9): Xaa is any amino acid except M, P and R
VECTMVEKXVLALLDKPPFLTQLHS

SEQ ID NO: 24 - protein, 13 aa, artificial sequence
  mutated segment of kinase domain of alphaPKC
  MISC_FEATURE (6)..(6): Xaa is any amino acid derivative suitable for stapling
  MISC_FEATURE (13)..(13): Xaa is any amino acid derivative suitable for stapling
VECTMXEKRVLAX

SEQ ID NO: 25 - protein, 13 aa, artificial sequence
  mutated segment of kinase domain of alphaPKC
  MISC_FEATURE (5)..(5): Xaa is any amino acid except M, P and R
  MISC_FEATURE (6)..(6): Xaa is any amino acid derivative suitable for stapling
  MISC_FEATURE (13)..(13): Xaa is any amino acid derivative suitable for stapling
VECTXXEKRVLAX

SEQ ID NO: 26 - protein, 13 aa, artificial sequence
  mutated segment of kinase domain of alphaPKC
  MISC_FEATURE (6)..(6): Xaa is any amino acid derivative suitable for stapling
  MISC_FEATURE (9)..(9): Xaa is any amino acid except M, P and R
  MISC_FEATURE (13)..(13): Xaa is any amino acid derivative suitable for stapling
VECTMXEKXVLAX

SEQ ID NO: 27 - protein, 13 aa, artificial sequence
  mutated segment of kinase domain of alphaPKC
  MISC_FEATURE (5)..(5): Xaa is any amino acid except M, P and R
  MISC_FEATURE (6)..(6): Xaa is any amino acid derivative suitable for stapling
  MISC_FEATURE (9)..(9): Xaa is any amino acid except M, P and R
  MISC_FEATURE (13)..(13): Xaa is any amino acid derivative suitable for stapling
VECTXXEKXVLAX

SEQ ID NO: 28 - protein, 25 aa, artificial sequence
  mutated segment of kinase domain of alphaPKC
  MISC_FEATURE (5)..(5): Xaa is any amino acid except M, P and R
  MISC_FEATURE (6)..(6): Xaa is any amino acid derivative suitable for stapling
  MISC_FEATURE (9)..(9): Xaa is any amino acid except M, P and R
  MISC_FEATURE (13)..(13): Xaa is any amino acid derivative suitable for stapling
  MISC_FEATURE (17)..(18): Xaa is any amino acid except M, P and R
VECTXXEKXVLAXLDKXXFLTQLHS

SEQ ID NO: 29 - protein, 25 aa, artificial sequence
  mutated segment of kinase domain of alphaPKC
  MISC_FEATURE (6)..(6): Xaa is any amino acid derivative suitable for stapling
  MISC_FEATURE (13)..(13): Xaa is any amino acid derivative suitable for stapling
  MISC_FEATURE (17)..(18): Xaa is any amino acid except M, P and R
VECTMXEKRVLAXLDKXXFLTQLHS

SEQ ID NO: 30 - protein, 25 aa, artificial sequence
  mutated segment of kinase domain of alphaPKC
  MISC_FEATURE (5)..(5): Xaa is any amino acid except M, P and R
  MISC_FEATURE (6)..(6): Xaa is any amino acid derivative suitable for stapling
  MISC_FEATURE (13)..(13): Xaa is any amino acid derivative suitable for stapling
VECTXXEKRVLAXLDKPPFLTQLHS

SEQ ID NO: 31 - protein, 25 aa, artificial sequence
  mutated segment of kinase domain of alphaPKC
  MISC_FEATURE (6)..(6): Xaa is any amino acid derivative suitable for stapling
  MISC_FEATURE (9)..(9): Xaa is any amino acid except M, P and R
  MISC_FEATURE (13)..(13): Xaa is any amino acid derivative suitable for stapling
VECTMXEKXVLAXLDKPPFLTQLHS

SEQ ID NO: 32 - protein, 25 aa, artificial sequence
  mutated segment of kinase domain of alphaPKC
VECTTREKEVLASLDKAAFLTQLHS

SEQ ID NO: 33 - protein, 8 aa, artificial sequence
  protein transduction domain
RRRRRRRR

SEQ ID NO: 34 - protein, 15 aa, artificial sequence
  protein transduction domain
RRPRRPRRPRRPRRP

SEQ ID NO: 35 - protein, 16 aa, artificial sequence
  penetratin peptide
RQIKIWFQNRRMKWKK

SEQ ID NO: 36 - protein, 11 aa, artificial sequence
  HIV-tat
YGRKKRRQRRR

SEQ ID NO: 37 - DNA, 20 bp, artificial sequence
  primer
tgctttggtttctgggactt

SEQ ID NO: 38 - DNA, 20 bp, artificial sequence
  primer
gctctagccgaacacgaatc

SEQ ID NO: 39 - DNA, 22 bp, artificial sequence
  primer
tggacaaagtagacggagtgtc

SEQ ID NO: 40 - DNA, 20 bp, artificial sequence
  primer
tagcaaggcctgtcccatac

SEQ ID NO: 41 - DNA, 20 bp, artificial sequence
  primer
tgagaacttgccaccgtatg

SEQ ID NO: 42 - DNA, 20 bp, artificial sequence
  primer
ggcaggtaggcccctatatc

SEQ ID NO: 43 - DNA, 20 bp, artificial sequence
  primer
gtttcatccgggtcttcatc

SEQ ID NO: 44 - DNA, 20 bp, artificial sequence
  primer
gtgtctgtgccctcgaaaat

SEQ ID NO: 45 - DNA, 20 bp, artificial sequence
  primer
aagttctctgcctcccgatt

SEQ ID NO: 46 - DNA, 20 bp, artificial sequence
  primer
caaagcgttgctggaagttt

SEQ ID NO: 47 - DNA, 20 bp, artificial sequence
  primer
tcgattccctcctacactgc

SEQ ID NO: 48 - DNA, 20 bp, artificial sequence
  primer
ttggtggtactggctcatca

SEQ ID NO: 49 - protein, 25 aa, ARTIFICIAL
  Stapled peptide sequence A
  MISC_FEATURE (6)..(6): Xaa is any amino acid derivative suitable for stapling
  MISC_FEATURE (13)..(13): Xaa is any amino acid derivative suitable for stapling
VECTMXEKRVLAXLDKPPFLTQLHS

SEQ ID NO: 50 - protein, 21 aa, artificial
  Stapled peptide sequence B
  MISC_FEATURE (2)..(2): Xaa is any amino acid derivative suitable for stapling
  MISC_FEATURE (9)..(9): Xaa is any amino acid derivative suitable for stapling
SXCKGLMTXHPAKRLGCGPEG

SEQ ID NO: 51 - protein, 26 aa, artificial
  Scrambled peptide sequence A
KEVPVDTCHLTLMLLFRSVALKQHPE

SEQ ID NO: 52 - protein, 21 aa, artificial
  Scrambled peptide sequence B
SAECKGRHGTPPGKLMICKGL